European Patent Application EP 4 722 256 A1, published April 8, 2026. Title: 一种新型小型化CAR分子设计及制备方法和应用. Applicant: 四川大学华西医院. The sequence listing filed with the application follows.

SEQUENCE LISTING (18 sequences)

SEQ ID NO: 1 - DNA, 846 bp, synthetic construct
  source 1..846: mol_type = other DNA
atggccttaccagtgaccgccttgctcctgccgctggccttgctgctccacgccgccaggccggaggtgcagctggtggagagcggggggggactggtgcaggcaggaggaagcctgagactgagctgtgccgcaagcgggattacatttagtatcaacacaatgggatggtacaggcaggctcctggcaagcagagagagctggtggctctgatttcaagcatcggagacacctactacgccgactctgtgaaaggacggttcaccatcagcagagacaacgcaaagaacaccgtctacctgcagatgaacagcctgaaacctgaagacacagcagtgtactattgcaaaaggttccgaaccgctgctcagggcactgactactggggccagggcacccaggtgaccgtgtccagcaccacgacgccagcgccgcgaccaccaacaccggcgcccaccatcgcgtcgcagcccctgtccctgcgcccagaggcgtgccggccagcggcggggggcgcagtgcacacgagggggctggacttcgcctgtgatatctacatctgggcgcccctggccgggacttgtggggtccttctcctgtcactggttatcaccaaacggggcagaaagaaactcctgtatatattcaaacaaccatttatgagaccagtacaaactactcaagaggaagatggctgtagctgccgatttccagaagaagaagaaggaggatgtgaactggcccccgcgtaccagcagggccagaaccagctctataacgagctcaatctaggacgaagagaggagtacgatgttttgcacatgcaggccctgccccctcgctga

SEQ ID NO: 2 - DNA, 102 bp, synthetic construct
  source 1..102: mol_type = other DNA
gcccccgcgtaccagcagggccagaaccagctctataacgagctcaatctaggacgaagagaggagtacgatgttttgcacatgcaggccctgccccctcgc

SEQ ID NO: 3 - DNA, 354 bp, synthetic construct
  source 1..354: mol_type = other DNA
gaggtgcagctggtggagagcggggggggactggtgcaggcaggaggaagcctgagactgagctgtgccgcaagcgggattacatttagtatcaacacaatgggatggtacaggcaggctcctggcaagcagagagagctggtggctctgatttcaagcatcggagacacctactacgccgactctgtgaaaggacggttcaccatcagcagagacaacgcaaagaacaccgtctacctgcagatgaacagcctgaaacctgaagacacagcagtgtactattgcaaaaggttccgaaccgctgctcagggcactgactactggggccagggcacccaggtgaccgtgtccagc

SEQ ID NO: 4 - DNA, 198 bp, synthetic construct
  source 1..198: mol_type = other DNA
accacgacgccagcgccgcgaccaccaacaccggcgcccaccatcgcgtcgcagcccctgtccctgcgcccagaggcgtgccggccagcggcggggggcgcagtgcacacgagggggctggacttcgcctgtgatatctacatctgggcgcccctggccgggacttgtggggtccttctcctgtcactggttatcacc

SEQ ID NO: 5 - DNA, 849 bp, synthetic construct
  source 1..849: mol_type = other DNA
atggccttaccagtgaccgccttgctcctgccgctggccttgctgctccacgccgccaggccgcaggtccagctggtcgagtctggaggtggcctggtccagccaggtggcagtctgaggctgagttgcgcagcctctggagtggacatctcttccgacgtgatggcctggtataggcaggcacctggtaagggactggaatttgtctctggtctgactagaggtggcagcatcaactacgctgacagcgtcaagggaaggtttaccatcagcagggacaactccaagaacaccttgtacctgcagatgaacagcctgagagccgaagatacagccgtgtactactgcaacgccgaaatctacaccggcaccttctacccacggtcttactggggccagggcacattggtaaccgtgtcaaccacgacgccagcgccgcgaccaccaacaccggcgcccaccatcgcgtcgcagcccctgtccctgcgcccagaggcgtgccggccagcggcggggggcgcagtgcacacgagggggctggacttcgcctgtgatatctacatctgggcgcccctggccgggacttgtggggtccttctcctgtcactggttatcaccaaacggggcagaaagaaactcctgtatatattcaaacaaccatttatgagaccagtacaaactactcaagaggaagatggctgtagctgccgatttccagaagaagaagaaggaggatgtgaactggcccccgcgtaccagcagggccagaaccagctctataacgagctcaatctaggacgaagagaggagtacgatgttttgcacatgcaggccctgccccctcgctga

SEQ ID NO: 6 - DNA, 357 bp, synthetic construct
  source 1..357: mol_type = other DNA
caggtccagctggtcgagtctggaggtggcctggtccagccaggtggcagtctgaggctgagttgcgcagcctctggagtggacatctcttccgacgtgatggcctggtataggcaggcacctggtaagggactggaatttgtctctggtctgactagaggtggcagcatcaactacgctgacagcgtcaagggaaggtttaccatcagcagggacaactccaagaacaccttgtacctgcagatgaacagcctgagagccgaagatacagccgtgtactactgcaacgccgaaatctacaccggcaccttctacccacggtcttactggggccagggcacattggtaaccgtgtca

SEQ ID NO: 7 - DNA, 885 bp, synthetic construct
  source 1..885: mol_type = other DNA
atggccctgcctgttacagctctgctgctgcctctggctctgcttctgcatgccgccagacctgaggtgcagctgttggagtctgggggaggcttggtacagcctggggggtccctgagactctcctgtgcagcctctggattcacctttagcagctatgccatgagctgggtccgccaggctccagggaaggggctggagtgggtctcatctattagtggtagtggtgattacatatactacgcagactccgtgaagggccggttcaccatctccagagacatatccaagaacacgctgtatctgcaaatgaacagcctgagagccgaggacacggccgtatattactgtgcgaaagaaggtacgggtgccaacagcagcttggcagactacagaggccagggcaccctggtcaccgtctcctcattcgtgcccgtgttcctgcctgccaagcctaccacgacgccagcgccgcgaccaccaacaccggcgcccaccatcgcgtcgcagcccctgtccctgcgcccagaggcgtgccggccagcggcggggggcgcagtgcacacgagggggctggacttcgcctgtgatatctacatctgggcgcccctggccgggacttgtggggtccttctcctgtcactggttatcaccaaacggggcagaaagaaactcctgtatatattcaaacaaccatttatgagaccagtacaaactactcaagaggaagatggctgtagctgccgatttccagaagaagaagaaggaggatgtgaactggcccccgcgtaccagcagggccagaaccagctctataacgagctcaatctaggacgaagagaggagtacgatgttttgcacatgcaggccctgccccctcgctga

SEQ ID NO: 8 - DNA, 393 bp, synthetic construct
  source 1..393: mol_type = other DNA
gaggtgcagctgttggagtctgggggaggcttggtacagcctggggggtccctgagactctcctgtgcagcctctggattcacctttagcagctatgccatgagctgggtccgccaggctccagggaaggggctggagtgggtctcatctattagtggtagtggtgattacatatactacgcagactccgtgaagggccggttcaccatctccagagacatatccaagaacacgctgtatctgcaaatgaacagcctgagagccgaggacacggccgtatattactgtgcgaaagaaggtacgggtgccaacagcagcttggcagactacagaggccagggcaccctggtcaccgtctcctcattcgtgcccgtgttcctgcctgccaagcct

SEQ ID NO: 9 - DNA, 846 bp, synthetic construct
  source 1..846: mol_type = other DNA
atggccttaccagtgaccgccttgctcctgccgctggccttgctgctccacgccgccaggccggaggtgcagctggtggagagcggggggggactggtgcaggcaggaggaagcctgagactgagctgtgccgcaagcgggattacatttagtatcaacacaatgggatggtacaggcaggctcctggcaagcagagagagctggtggctctgatttcaagcatcggagacacctactacgccgactctgtgaaaggacggttcaccatcagcagagacaacgcaaagaacaccgtctacctgcagatgaacagcctgaaacctgaagacacagcagtgtactattgcaaaaggttccgaaccgctgctcagggcactgactactggggccagggcacccaggtgaccgtgtccagcattgaagttatgtatcctcctccttacctagacaatgagaagagcaatggaaccattatccatgtgaaagggaaacacctttgtccaagtcccctatttcccggaccttctaagcccttttgggtgctggtggtggttggtggagtcctggcttgctatagcttgctagtaacagtggcctttattattttctgggtgaaacggggcagaaagaaactcctgtatatattcaaacaaccatttatgagaccagtacaaactactcaagaggaagatggctgtagctgccgatttccagaagaagaagaaggaggatgtgaactggcccccgcgtaccagcagggccagaaccagctctataacgagctcaatctaggacgaagagaggagtacgatgttttgcacatgcaggccctgccccctcgctga

SEQ ID NO: 10 - DNA, 198 bp, synthetic construct
  source 1..198: mol_type = other DNA
attgaagttatgtatcctcctccttacctagacaatgagaagagcaatggaaccattatccatgtgaaagggaaacacctttgtccaagtcccctatttcccggaccttctaagcccttttgggtgctggtggtggttggtggagtcctggcttgctatagcttgctagtaacagtggcctttattattttctgggtg

SEQ ID NO: 11 - DNA, 828 bp, synthetic construct
  source 1..828: mol_type = other DNA
atggccttaccagtgaccgccttgctcctgccgctggccttgctgctccacgccgccaggccggaggtgcagctggtggagagcggggggggactggtgcaggcaggaggaagcctgagactgagctgtgccgcaagcgggattacatttagtatcaacacaatgggatggtacaggcaggctcctggcaagcagagagagctggtggctctgatttcaagcatcggagacacctactacgccgactctgtgaaaggacggttcaccatcagcagagacaacgcaaagaacaccgtctacctgcagatgaacagcctgaaacctgaagacacagcagtgtactattgcaaaaggttccgaaccgctgctcagggcactgactactggggccagggcacccaggtgaccgtgtccagcattgaagttatgtatcctcctccttacctagacaatgagaagagcaatggaaccattatccatgtgaaagggaaacacctttgtccaagtcccctatttcccggaccttctaagcccctctgctacctgctggatggaatcctcttcatctatggtgtcattctcactgccttgttcctgaaacggggcagaaagaaactcctgtatatattcaaacaaccatttatgagaccagtacaaactactcaagaggaagatggctgtagctgccgatttccagaagaagaagaaggaggatgtgaactggcccccgcgtaccagcagggccagaaccagctctataacgagctcaatctaggacgaagagaggagtacgatgttttgcacatgcaggccctgccccctcgctga

SEQ ID NO: 12 - DNA, 180 bp, synthetic construct
  source 1..180: mol_type = other DNA
attgaagttatgtatcctcctccttacctagacaatgagaagagcaatggaaccattatccatgtgaaagggaaacacctttgtccaagtcccctatttcccggaccttctaagcccctctgctacctgctggatggaatcctcttcatctatggtgtcattctcactgccttgttcctg

SEQ ID NO: 13 - DNA, 846 bp, synthetic construct
  source 1..846: mol_type = other DNA
atggccttaccagtgaccgccttgctcctgccgctggccttgctgctccacgccgccaggccggaggtgcagctggtggagagcggggggggactggtgcaggcaggaggaagcctgagactgagctgtgccgcaagcgggattacatttagtatcaacacaatgggatggtacaggcaggctcctggcaagcagagagagctggtggctctgatttcaagcatcggagacacctactacgccgactctgtgaaaggacggttcaccatcagcagagacaacgcaaagaacaccgtctacctgcagatgaacagcctgaaacctgaagacacagcagtgtactattgcaaaaggttccgaaccgctgctcagggcactgactactggggccagggcacccaggtgaccgtgtccagcaccacgacgccagcgccgcgaccaccaacaccggcgcccaccatcgcgtcgcagcccctgtccctgcgcccagaggcgtgccggccagcggcggggggcgcagtgcacacgagggggctggacttcgcctgtgatctctgctacctgctggatggaatcctcttcatctatggtgtcattctcactgccttgttcctgaaacggggcagaaagaaactcctgtatatattcaaacaaccatttatgagaccagtacaaactactcaagaggaagatggctgtagctgccgatttccagaagaagaagaaggaggatgtgaactggcccccgcgtaccagcagggccagaaccagctctataacgagctcaatctaggacgaagagaggagtacgatgttttgcacatgcaggccctgccccctcgctga

SEQ ID NO: 14 - DNA, 198 bp, synthetic construct
  source 1..198: mol_type = other DNA
accacgacgccagcgccgcgaccaccaacaccggcgcccaccatcgcgtcgcagcccctgtccctgcgcccagaggcgtgccggccagcggcggggggcgcagtgcacacgagggggctggacttcgcctgtgatctctgctacctgctggatggaatcctcttcatctatggtgtcattctcactgccttgttcctg

SEQ ID NO: 15 - DNA, 1218 bp, synthetic construct
  source 1..1218: mol_type = other DNA
atggccttaccagtgaccgccttgctcctgccgctggccttgctgctccacgccgccaggccgatgcaggtacaactgcagcagtcaggacctgaactgaagaagcctggagagacagtcaagatctcctgcaaggcctctgggtatcctttcacaaactatggaatgaactgggtgaagcaggctccaggacagggtttaaagtggatgggctggattaacacctccactggagagtcaacatttgctgatgacttcaagggacggtttgacttctctttggaaacctctgccaacactgcctatttgcagatcaacaacctcaaaagtgaagactcggctacatatttctgtgcaagatgggaggtttaccacggctacgttccttactggggccaagggaccacggtcaccgtttcctctggcggtggcggttctggtggcggtggctccggcggtggcggttctgacatccagctgacccagtctcacaaattcctgtccacttcagtaggagacagggtcagcatcacctgcaaggccagtcaggatgtgtataatgctgttgcctggtatcaacagaaaccaggacaatctcctaaacttctgatttactcggcatcctcccggtacactggagtcccttctcgcttcactggcagtggctctgggccggatttcactttcaccatcagcagtgtgcaggctgaagacctggcagtttatttctgtcagcaacattttcgtactccattcacgttcggctcggggacaaaattggagatcaaaaccacgacgccagcgccgcgaccaccaacaccggcgcccaccatcgcgtcgcagcccctgtccctgcgcccagaggcgtgccggccagcggcggggggcgcagtgcacacgagggggctggacttcgcctgtgatatctacatctgggcgcccctggccgggacttgtggggtccttctcctgtcactggttatcaccaaacggggcagaaagaaactcctgtatatattcaaacaaccatttatgagaccagtacaaactactcaagaggaagatggctgtagctgccgatttccagaagaagaagaaggaggatgtgaactggcccccgcgtaccagcagggccagaaccagctctataacgagctcaatctaggacgaagagaggagtacgatgttttgcacatgcaggccctgccccctcgctga

SEQ ID NO: 16 - DNA, 726 bp, synthetic construct
  source 1..726: mol_type = other DNA
atgcaggtacaactgcagcagtcaggacctgaactgaagaagcctggagagacagtcaagatctcctgcaaggcctctgggtatcctttcacaaactatggaatgaactgggtgaagcaggctccaggacagggtttaaagtggatgggctggattaacacctccactggagagtcaacatttgctgatgacttcaagggacggtttgacttctctttggaaacctctgccaacactgcctatttgcagatcaacaacctcaaaagtgaagactcggctacatatttctgtgcaagatgggaggtttaccacggctacgttccttactggggccaagggaccacggtcaccgtttcctctggcggtggcggttctggtggcggtggctccggcggtggcggttctgacatccagctgacccagtctcacaaattcctgtccacttcagtaggagacagggtcagcatcacctgcaaggccagtcaggatgtgtataatgctgttgcctggtatcaacagaaaccaggacaatctcctaaacttctgatttactcggcatcctcccggtacactggagtcccttctcgcttcactggcagtggctctgggccggatttcactttcaccatcagcagtgtgcaggctgaagacctggcagtttatttctgtcagcaacattttcgtactccattcacgttcggctcggggacaaaattggagatcaaa

SEQ ID NO: 17 - DNA, 1428 bp, synthetic construct
  source 1..1428: mol_type = other DNA
atggccttaccagtgaccgccttgctcctgccgctggccttgctgctccacgccgccaggccgatgcaggtacaactgcagcagtcaggacctgaactgaagaagcctggagagacagtcaagatctcctgcaaggcctctgggtatcctttcacaaactatggaatgaactgggtgaagcaggctccaggacagggtttaaagtggatgggctggattaacacctccactggagagtcaacatttgctgatgacttcaagggacggtttgacttctctttggaaacctctgccaacactgcctatttgcagatcaacaacctcaaaagtgaagactcggctacatatttctgtgcaagatgggaggtttaccacggctacgttccttactggggccaagggaccacggtcaccgtttcctctggcggtggcggttctggtggcggtggctccggcggtggcggttctgacatccagctgacccagtctcacaaattcctgtccacttcagtaggagacagggtcagcatcacctgcaaggccagtcaggatgtgtataatgctgttgcctggtatcaacagaaaccaggacaatctcctaaacttctgatttactcggcatcctcccggtacactggagtcccttctcgcttcactggcagtggctctgggccggatttcactttcaccatcagcagtgtgcaggctgaagacctggcagtttatttctgtcagcaacattttcgtactccattcacgttcggctcggggacaaaattggagatcaaaaccacgacgccagcgccgcgaccaccaacaccggcgcccaccatcgcgtcgcagcccctgtccctgcgcccagaggcgtgccggccagcggcggggggcgcagtgcacacgagggggctggacttcgcctgtgatatctacatctgggcgcccctggccgggacttgtggggtccttctcctgtcactggttatcaccaaacggggcagaaagaaactcctgtatatattcaaacaaccatttatgagaccagtacaaactactcaagaggaagatggctgtagctgccgatttccagaagaagaagaaggaggatgtgaactggcccccgcgtaccagcagggccagaaccagctctataacgagctcaatctaggacgaagagaggagtacgatgttttggacaagagacgtggccgggaccctgagatggggggaaagccgcagagaaggaagaaccctcaggaaggcctgtacaatgaactgcagaaagataagatggcggaggcctacagtgagattgggatgaaaggcgagcgccggaggggcaaggggcacgatggcctttaccagggtctcagtacagccaccaaggacacctacgacgcccttcacatgcaggccctgccccctcgctga

SEQ ID NO: 18 - DNA, 312 bp, synthetic construct
  source 1..312: mol_type = other DNA
gcccccgcgtaccagcagggccagaaccagctctataacgagctcaatctaggacgaagagaggagtacgatgttttggacaagagacgtggccgggaccctgagatggggggaaagccgcagagaaggaagaaccctcaggaaggcctgtacaatgaactgcagaaagataagatggcggaggcctacagtgagattgggatgaaaggcgagcgccggaggggcaaggggcacgatggcctttaccagggtctcagtacagccaccaaggacacctacgacgcccttcacatgcaggccctgccccctcgc